European Patent Application EP 4 202 046 A1, published June 28, 2023. Title: POLYNUCLEOTIDE HAVING PROMOTER ACTIVITY AND APPLICATION OF POLYNUCLEOTIDE IN PRODUCING AMINO ACID. Applicant: Tianjin Institute of Industrial Biotechnology, Chinese Academy of Sciences. The sequence listing filed with the application follows.

SEQUENCE LISTING (38 sequences)

SEQ ID NO: 1 - DNA, 42 bp, Corynebacterium glutamicum
cctgatgcggtattttctccgtgcgtggcgagttttacaaag

SEQ ID NO: 2 - DNA, 21 bp, Corynebacterium glutamicum
gacgtcgcgtgcgatcagatc

SEQ ID NO: 3 - DNA, 84 bp, Plasmid
atctgatcgcacgcgacgtcggcggtggctctggaggtggtgggtccggcggtggctctgcttcctccgaagacgttatcaaag

SEQ ID NO: 4 - DNA, 21 bp, Plasmid
ggagaaaataccgcatcaggc

SEQ ID NO: 5 - DNA, 51 bp, Corynebacterium glutamicum
ccctgaatcatcatctaagtnnnnnnnnnggtaagctcgaccaggacagtg

SEQ ID NO: 6 - DNA, 25 bp, Corynebacterium glutamicum
aaccttccatacgaactttgaaacg

SEQ ID NO: 7 - DNA, 23 bp, Corynebacterium glutamicum
caaagttcgtatggaaggttccg

SEQ ID NO: 8 - DNA, 22 bp, Corynebacterium glutamicum
acttagatgatgattcagggac

SEQ ID NO: 9 - DNA, 351 bp, Corynebacterium glutamicum
gtgcgtggcgagttttacaaagaaccccacatcatcaatgcctaaatggcgggtattttcatccaaacccaaccgcgcatcattccaatgctgatccaccccatccggataaaccaccatgaacggcaacggatcaaaagtcctgttggtgaagctgcgccccacagatcctgactgctgggagccatgaaaatagatcagcgcatccgtggtggaaccaaaaggctcaacaatacgaaacgttcgctttcggtcctgatgaaagagatgtccctgaatcatcatctaagtatgcatctcggtaagctcgaccaggacagtgccaccacaattttggaggattacaagaac

SEQ ID NO: 10 - DNA, 351 bp, Corynebacterium glutamicum
gtgcgtggcgagttttacaaagaaccccacatcatcaatgcctaaatggcgggtattttcatccaaacccaaccgcgcatcattccaatgctgatccaccccatccggataaaccaccatgaacggcaacggatcaaaagtcctgttggtgaagctgcgccccacagatcctgactgctgggagccatgaaaatagatcagcgcatccgtggtggaaccaaaaggctcaacaatacgaaacgttcgctttcggtcctgatgaaagagatgtccctgaatcatcatctaagtacaaaaggtggtaagctcgaccaggacagtgccaccacaattttggaggattacaagaac

SEQ ID NO: 11 - DNA, 351 bp, Corynebacterium glutamicum
gtgcgtggcgagttttacaaagaaccccacatcatcaatgcctaaatggcgggtattttcatccaaacccaaccgcgcatcattccaatgctgatccaccccatccggataaaccaccatgaacggcaacggatcaaaagtcctgttggtgaagctgcgccccacagatcctgactgctgggagccatgaaaatagatcagcgcatccgtggtggaaccaaaaggctcaacaatacgaaacgttcgctttcggtcctgatgaaagagatgtccctgaatcatcatctaagttcttcatctggtaagctcgaccaggacagtgccaccacaattttggaggattacaagaac

SEQ ID NO: 12 - DNA, 351 bp, Corynebacterium glutamicum
gtgcgtggcgagttttacaaagaaccccacatcatcaatgcctaaatggcgggtattttcatccaaacccaaccgcgcatcattccaatgctgatccaccccatccggataaaccaccatgaacggcaacggatcaaaagtcctgttggtgaagctgcgccccacagatcctgactgctgggagccatgaaaatagatcagcgcatccgtggtggaaccaaaaggctcaacaatacgaaacgttcgctttcggtcctgatgaaagagatgtccctgaatcatcatctaagtggaaagtatggtaagctcgaccaggacagtgccaccacaattttggaggattacaagaac

SEQ ID NO: 13 - DNA, 351 bp, Corynebacterium glutamicum
gtgcgtggcgagttttacaaagaaccccacatcatcaatgcctaaatggcgggtattttcatccaaacccaaccgcgcatcattccaatgctgatccaccccatccggataaaccaccatgaacggcaacggatcaaaagtcctgttggtgaagctgcgccccacagatcctgactgctgggagccatgaaaatagatcagcgcatccgtggtggaaccaaaaggctcaacaatacgaaacgttcgctttcggtcctgatgaaagagatgtccctgaatcatcatctaagtttattatatggtaagctcgaccaggacagtgccaccacaattttggaggattacaagaac

SEQ ID NO: 14 - DNA, 351 bp, Corynebacterium glutamicum
gtgcgtggcgagttttacaaagaaccccacatcatcaatgcctaaatggcgggtattttcatccaaacccaaccgcgcatcattccaatgctgatccaccccatccggataaaccaccatgaacggcaacggatcaaaagtcctgttggtgaagctgcgccccacagatcctgactgctgggagccatgaaaatagatcagcgcatccgtggtggaaccaaaaggctcaacaatacgaaacgttcgctttcggtcctgatgaaagagatgtccctgaatcatcatctaagttaatcctctggtaagctcgaccaggacagtgccaccacaattttggaggattacaagaac

SEQ ID NO: 15 - DNA, 351 bp, Corynebacterium glutamicum
gtgcgtggcgagttttacaaagaaccccacatcatcaatgcctaaatggcgggtattttcatccaaacccaaccgcgcatcattccaatgctgatccaccccatccggataaaccaccatgaacggcaacggatcaaaagtcctgttggtgaagctgcgccccacagatcctgactgctgggagccatgaaaatagatcagcgcatccgtggtggaaccaaaaggctcaacaatacgaaacgttcgctttcggtcctgatgaaagagatgtccctgaatcatcatctaagttcaatttatggtaagctcgaccaggacagtgccaccacaattttggaggattacaagaac

SEQ ID NO: 16 - DNA, 351 bp, Corynebacterium glutamicum
gtgcgtggcgagttttacaaagaaccccacatcatcaatgcctaaatggcgggtattttcatccaaacccaaccgcgcatcattccaatgctgatccaccccatccggataaaccaccatgaacggcaacggatcaaaagtcctgttggtgaagctgcgccccacagatcctgactgctgggagccatgaaaatagatcagcgcatccgtggtggaaccaaaaggctcaacaatacgaaacgttcgctttcggtcctgatgaaagagatgtccctgaatcatcatctaagtgcgcaatctggtaagctcgaccaggacagtgccaccacaattttggaggattacaagaac

SEQ ID NO: 17 - DNA, 351 bp, Corynebacterium glutamicum
gtgcgtggcgagttttacaaagaaccccacatcatcaatgcctaaatggcgggtattttcatccaaacccaaccgcgcatcattccaatgctgatccaccccatccggataaaccaccatgaacggcaacggatcaaaagtcctgttggtgaagctgcgccccacagatcctgactgctgggagccatgaaaatagatcagcgcatccgtggtggaaccaaaaggctcaacaatacgaaacgttcgctttcggtcctgatgaaagagatgtccctgaatcatcatctaagtcagttccgtggtaagctcgaccaggacagtgccaccacaattttggaggattacaagaac

SEQ ID NO: 18 - DNA, 351 bp, Corynebacterium glutamicum
gtgcgtggcgagttttacaaagaaccccacatcatcaatgcctaaatggcgggtattttcatccaaacccaaccgcgcatcattccaatgctgatccaccccatccggataaaccaccatgaacggcaacggatcaaaagtcctgttggtgaagctgcgccccacagatcctgactgctgggagccatgaaaatagatcagcgcatccgtggtggaaccaaaaggctcaacaatacgaaacgttcgctttcggtcctgatgaaagagatgtccctgaatcatcatctaagtaagttttatggtaagctcgaccaggacagtgccaccacaattttggaggattacaagaac

SEQ ID NO: 19 - DNA, 351 bp, Corynebacterium glutamicum
gtgcgtggcgagttttacaaagaaccccacatcatcaatgcctaaatggcgggtattttcatccaaacccaaccgcgcatcattccaatgctgatccaccccatccggataaaccaccatgaacggcaacggatcaaaagtcctgttggtgaagctgcgccccacagatcctgactgctgggagccatgaaaatagatcagcgcatccgtggtggaaccaaaaggctcaacaatacgaaacgttcgctttcggtcctgatgaaagagatgtccctgaatcatcatctaagttaaatgtatggtaagctcgaccaggacagtgccaccacaattttggaggattacaagaac

SEQ ID NO: 20 - DNA, 351 bp, Corynebacterium glutamicum
gtgcgtggcgagttttacaaagaaccccacatcatcaatgcctaaatggcgggtattttcatccaaacccaaccgcgcatcattccaatgctgatccaccccatccggataaaccaccatgaacggcaacggatcaaaagtcctgttggtgaagctgcgccccacagatcctgactgctgggagccatgaaaatagatcagcgcatccgtggtggaaccaaaaggctcaacaatacgaaacgttcgctttcggtcctgatgaaagagatgtccctgaatcatcatctaagtggattgtatggtaagctcgaccaggacagtgccaccacaattttggaggattacaagaac

SEQ ID NO: 21 - DNA, 351 bp, Corynebacterium glutamicum
gtgcgtggcgagttttacaaagaaccccacatcatcaatgcctaaatggcgggtattttcatccaaacccaaccgcgcatcattccaatgctgatccaccccatccggataaaccaccatgaacggcaacggatcaaaagtcctgttggtgaagctgcgccccacagatcctgactgctgggagccatgaaaatagatcagcgcatccgtggtggaaccaaaaggctcaacaatacgaaacgttcgctttcggtcctgatgaaagagatgtccctgaatcatcatctaagtcaaactcatggtaagctcgaccaggacagtgccaccacaattttggaggattacaagaac

SEQ ID NO: 22 - DNA, 351 bp, Corynebacterium glutamicum
gtgcgtggcgagttttacaaagaaccccacatcatcaatgcctaaatggcgggtattttcatccaaacccaaccgcgcatcattccaatgctgatccaccccatccggataaaccaccatgaacggcaacggatcaaaagtcctgttggtgaagctgcgccccacagatcctgactgctgggagccatgaaaatagatcagcgcatccgtggtggaaccaaaaggctcaacaatacgaaacgttcgctttcggtcctgatgaaagagatgtccctgaatcatcatctaagttacaaatctggtaagctcgaccaggacagtgccaccacaattttggaggattacaagaac

SEQ ID NO: 23 - DNA, 351 bp, Corynebacterium glutamicum
gtgcgtggcgagttttacaaagaaccccacatcatcaatgcctaaatggcgggtattttcatccaaacccaaccgcgcatcattccaatgctgatccaccccatccggataaaccaccatgaacggcaacggatcaaaagtcctgttggtgaagctgcgccccacagatcctgactgctgggagccatgaaaatagatcagcgcatccgtggtggaaccaaaaggctcaacaatacgaaacgttcgctttcggtcctgatgaaagagatgtccctgaatcatcatctaagttatcagtctggtaagctcgaccaggacagtgccaccacaattttggaggattacaagaac

SEQ ID NO: 24 - DNA, 351 bp, Corynebacterium glutamicum
gtgcgtggcgagttttacaaagaaccccacatcatcaatgcctaaatggcgggtattttcatccaaacccaaccgcgcatcattccaatgctgatccaccccatccggataaaccaccatgaacggcaacggatcaaaagtcctgttggtgaagctgcgccccacagatcctgactgctgggagccatgaaaatagatcagcgcatccgtggtggaaccaaaaggctcaacaatacgaaacgttcgctttcggtcctgatgaaagagatgtccctgaatcatcatctaagtcgaggatatggtaagctcgaccaggacagtgccaccacaattttggaggattacaagaac

SEQ ID NO: 25 - DNA, 351 bp, Corynebacterium glutamicum
gtgcgtggcgagttttacaaagaaccccacatcatcaatgcctaaatggcgggtattttcatccaaacccaaccgcgcatcattccaatgctgatccaccccatccggataaaccaccatgaacggcaacggatcaaaagtcctgttggtgaagctgcgccccacagatcctgactgctgggagccatgaaaatagatcagcgcatccgtggtggaaccaaaaggctcaacaatacgaaacgttcgctttcggtcctgatgaaagagatgtccctgaatcatcatctaagtccttgttatggtaagctcgaccaggacagtgccaccacaattttggaggattacaagaac

SEQ ID NO: 26 - DNA, 41 bp, Corynebacterium glutamicum
caggaaacagctatgacatgttccagccatcgccaaataag

SEQ ID NO: 27 - DNA, 22 bp, Corynebacterium glutamicum
acttagatgatgattcagggac

SEQ ID NO: 28 - DNA, 51 bp, Corynebacterium glutamicum
ccctgaatcatcatctaagtacaaaaggtggtaagctcgaccaggacagtg

SEQ ID NO: 29 - DNA, 51 bp, Corynebacterium glutamicum
ccctgaatcatcatctaagttaaatgtatggtaagctcgaccaggacagtg

SEQ ID NO: 30 - DNA, 51 bp, Corynebacterium glutamicum
ccctgaatcatcatctaagtccttgttatggtaagctcgaccaggacagtg

SEQ ID NO: 31 - DNA, 43 bp, Corynebacterium glutamicum
tgtaaaacgacggccagtgctgtactggactgccttttgaacg

SEQ ID NO: 32 - DNA, 19 bp, Plasmid
gcactggccgtcgttttac

SEQ ID NO: 33 - DNA, 24 bp, Plasmid
catgtcatagctgtttcctgtgtg

SEQ ID NO: 34 - DNA, 1331 bp, Corynebacterium glutamicum
cctgatgcggtattttctccgtgcgtggcgagttttacaaagaaccccacatcatcaatgcctaaatggcgggtattttcatccaaacccaaccgcgcatcattccaatgctgatccaccccatccggataaaccaccatgaacggcaacggatcaaaagtcctgttggtgaagctgcgccccacagatcctgactgctgggagccatgaaaatagatcagcgcatccgtggtggaaccaaaaggctcaacaatacgaaacgttcgctttcggtcctgatgaaagagatgtccctgaatcatcatctaagtatgcatctcggtaagctcgaccaggacagtgccaccacaattttggaggattacaagaacatgaccaacatccgcgtagctatcgtgggctacggaaacctgggacgcagcgtcgaaaagcttattgccaagcagcccgacatggaccttgtaggaatcttctcgcgccgggccaccctcgacacaaagacgccagtctttgatgtcgccgacgtggacaagcacgccgacgacgtggacgtgctgttcctgtgcatgggctccgccaccgacatccctgagcaggcaccaaagttcgcgcagttcgcctgcaccgtagacacctacgacaaccaccgcgacatcccacgccaccgccaggtcatgaacgaagccgccaccgcagccggcaacgttgcactggtctctaccggctgggatccaggaatgttctccatcaaccgcgtctacgcagcggcagtcttagccgagcaccagcagcacaccttctggggcccaggtttgtcacagggccactccgatgctttgcgacgcatccctggcgttcaaaaggcagtccagtacaccctcccatccgaagacgccctggaaaaggcccgccgcggcgaagccggcgaccttaccggaaagcaaacccacaagcgccaatgcttcgtggttgccgacgcggccgatcacgagcgcatcgaaaacgacatccgcaccatgcctgattacttcgttggctacgaagtcgaagtcaacttcatcgacgaagcaaccttcgactccgagcacaccggcatgccacacggtggccacgtgattaccaccggcgacaccggtggcttcaaccacaccgtggaatacatcctcaagctggaccgaaacccagatttcaccgcttcctcacagatcgctttcggtcgcgcagctcaccgcatgaagcagcagggccaaagcggagctttcaccgtcctcgaagttgctccatacctgctctccccagagaacttggacgatctgatcgcacgcgacgtc

SEQ ID NO: 35 - DNA, 5938 bp, Plasmid
atctgatcgcacgcgacgtcggcggtggctctggaggtggtgggtccggcggtggctctgcttcctccgaagacgttatcaaagagttcatgcgtttcaaagttcgtatggaaggttccgttaacggtcacgagttcgaaatcgaaggtgaaggtgaaggtcgtccgtacgaaggtacccagaccgctaaactgaaagttaccaaaggtggtccgctgccgttcgcttgggacatcctgtccccgcagttccagtacggttccaaagcttacgttaaacacccggctgacatcccggactacctgaaactgtccttcccggaaggtttcaaatgggaacgtgttatgaacttcgaagacggtggtgttgttaccgttacccaggactcctccctgcaagacggtgagttcatctacaaagttaaactgcgtggtaccaacttcccgtccgacggtccggttatgcagaaaaaaaccatgggttgggaagcttccaccgaacgtatgtacccggaagacggtgctctgaaaggtgaaatcaaaatgcgtctgaaactgaaagacggtggtcactacgacgctgaagttaaaaccacctacatggctaaaaaaccggttcagctgccgggtgcttacaaaaccgacatcaaactggacatcacctcccacaacgaagactacaccatcgttgaacagtacgaacgtgctgaaggtcgtcactccaccggtgcttaactgcaggcatgcaagcttggctgttttggcggatgagagaagattttcagcctgatacagattaaatcagaacgcagaagcggtctgataaaacagaatttgcctggcggcagtagcgcggtggtcccacctgaccccatgccgaactcagaagtgaaacgccgtagcgccgatggtagtgtggggtctccccatgcgagagtagggaactgccaggcatcaaataaaacgaaaggctcagtcgaaagactgggcctttcgttttatctgttgtttgtcggtgaacgctctcctgagtaggacaaatccgccgggagcggatttgaacgttgcgaagcaacggcccggagggtggcgggcaggacgcccgccataaactgccaggcatcaaattaagcagaaggccatcctgacggatggcctttttgcgtttctacaaactctttttgtttatttttctaaatacattcaaatatgtatccgctcatgaattaattccgctagatgacgtgcggcttcgacctcctgggcgtggcgcttgttggcgcgctcgcggctggctgcggcacgacacgcgtctgagcagtattttgcgcgccgtcctcgtgggtcaggccggggtgggatcaggccaccgcagtaggcgcagctgatgcgatcctccactactgcgcgtcctcctggcgctgccgagcacgcagctcgtcggccagctcttcaaggtcggccacaagcgtttctaggtcgctcgcggcacttgcccagtcgcgtgatgctggcgcgtctgtcgtatcgagggcgcggaaaaatccgatcaccgtttttaaatcgacggcggcatcgagtgcgtcggactccagcgcgacatcggagagatccaccgctgatgcttcaggccagttttggtacttcgtcgtgaaggtcatgacaccattataacgaacgttcgttaaaaattctagccccaattctgataatttcttccggcactcctgcgaaaacctgcgagacttcttgcccagaaaaaacgccaagcgcagcggttaccgcactttttttccaggtgatttcaccctgaccagcgaagcggcactttagtgcatgaggtgtgcccctggtttcccctctttggagggttcaacccaaaaaagcacacaagcaaaaatgaaaatcatcatgagcaagttggtgcgaagcagcaacgcgctagctccaaaaaggtctccaggatctcgaggagatttttgagggggagggagtcgaggaagagccagagcagaaggcggggaaccgttctctgccgacagcgtgagccccccttaaaaatcaggccggggaggaaccggggagggatcagagctaggagcgagacaccctaaagggggggaaccgttttctgctgacggtgtttcgtttattagttttcagcccgtggatagcggagggtgagggcaagtgagagccagagcaaggacgggacccctaaaggggggaaccgttttctgctgacggtgtttcgtttattagttttcagcccgtggacggccgcgtttagcttccattccaagtgcctttctgacttgttggatgcgcctttcactgacacctagttcgcctgcaagctcacgagtcgagggatcagcaaccgattgagaacgggcatccaggatcgcagttttgacgcgaagttcgagcaactcgcctgtcatttctcggcgtttgtttgcttccgctaatcgctgtcgcgtctcctgcgcatacttactttctgggtcagcccatctgcgtgcattcgatgtagctgcgccccgtcgccccatcgtcgctagagctttccgccctcggctgctctgcgtttccacccgacgagcagggacgactggctggcctttagccacgtagccgcgcacacgacgcgccatcgtcaggcgatcacgcatggcgggaagatccggctcccggccgtctgcaccgaccgcctgggcaacgttgtacgccacttcatacgcgtcgatgatcttggcatcttttaggcgctcaccagcagctttgagctggtatcccacggtcaacgcgtggcgaaacgcggtctcgtcgcgcgctcgctctggatttgtccagagcactcgcacgccgtcgatcaggtcgccggacgcgtccagggcgctcggcaggctcgcgtccaaaatcgctagcgccttggcttctgcggtggcgcgttgtgccgcttcaatgcgggcgcgtccgctggaaaagtcctgctcaatgtactttttcggcttctgtgatccggtcatcgttcgagcaatctccattaggtcggccagccgatccacacgatcatgctggcagtgccatttataggctgtcggatcgtctgagacgtgcagcggccaccggctcagcctatgcgaaaaagcctggtcagcgccgaaaacacgagtcatttcttccgtcgttgcagccagcaggcgcatatttgggctggttttacctgctgcggcatacaccgggtcaatgagccagatgagctggcatttcccgctcagcggattcacgccgatccaagccggcgctttttctaggcgtgcccatttctctaaaatcgcgtagacctgcgggtttacgtgctcaatcttcccgccggcctggtggctgggcacatcgatgtcaagcacgatcaccgcggcatgttgcgcgtgcgtcagcgcaacgtactggcaccgcgtcagcgcttttgagccagcccggtagagctttggttgggtttcgccggtatccgggtttttaatccaggcgctcgcgaaatctcttgtcttgctgccctggaagctttcgcgtcccaggtgagcgagcagttcgcggcgatcttctgccgtccagccgcgtgagccgcagcgcatagcttcggggtgggtgtcgaacagatcggcggacaatttccacgcgctagctgtgactgtgtcctgcggatcggctagagtcatgtcttgagtgctttctcccagctgatgactgggggttagccgacgccctgtgagttcccgctcacggggcgttcaactttttcaggtatttgtgcagcttatcgtgttttcttcgtaaatgaacgcttaactaccttgttaaacgtggcaaataggcaggattgatggggatctagcttcacgctgccgcaagcactcagggcgcaagggctgctaaaggaagcggaacacgtagaaagccagtccgcagaaacggtgctgaccccggatgaatgtcagctactgggctatctggacaagggaaaacgcaagcgcaaagagaaagcaggtagcttgcagtgggcttacatggcgatagctagactgggcggttttatggacagcaagcgaaccggaattgccagctggggcgccctctggtaaggttgggaagccctgcaaagtaaactggatggctttcttgccgccaaggatctgatggcgcaggggatcaagatctgatcaagagacaggatgaggatcgtttcgcatgattgaacaagatggattgcacgcaggttctccggccgcttgggtggagaggctattcggctatgactgggcacaacagacaatcggctgctctgatgccgccgtgttccggctgtcagcgcaggggcgcccggttctttttgtcaagaccgacctgtccggtgccctgaatgaactccaagacgaggcagcgcggctatcgtggctggccacgacgggcgttccttgcgcagctgtgctcgacgttgtcactgaagcgggaagggactggctgctattgggcgaagtgccggggcaggatctcctgtcatctcaccttgctcctgccgagaaagtatccatcatggctgatgcaatgcggcggctgcatacgcttgatccggctacctgcccattcgaccaccaagcgaaacatcgcatcgagcgagcacgtactcggatggaagccggtcttgtcgatcaggatgatctggacgaagagcatcaggggctcgcgccagccgaactgttcgccaggctcaaggcgcggatgcccgacggcgaggatctcgtcgtgacccatggcgatgcctgcttgccgaatatcatggtggaaaatggccgcttttctggattcatcgactgtggccggctgggtgtggcggaccgctatcaggacatagcgttggctacccgtgatattgctgaagagcttggcggcgaatgggctgaccgcttcctcgtgctttacggtatcgccgctcccgattcgcagcgcatcgccttctatcgccttcttgacgagttcttctgagcgggactctggggttcgcggaatcatgaccaaaatcccttaacgtgagttttcgttccactgagcgtcagaccccgtagaaaagatcaaaggatcttcttgagatcctttttttctgcgcgtaatctgctgcttgcaaacaaaaaaaccaccgctaccagcggtggtttgtttgccggatcaagagctaccaactctttttccgaaggtaactggcttcagcagagcgcagataccaaatactgtccttctagtgtagccgtagttaggccaccacttcaagaactctgtagcaccgcctacatacctcgctctgctaatcctgttaccagtggctgctgccagtggcgataagtcgtgtcttaccgggttggactcaagacgatagttaccggataaggcgcagcggtcgggctgaacggggggttcgtgcacacagcccagcttggagcgaacgacctacaccgaactgagatacctacagcgtgagctatgagaaagcgccacgcttcccgaagggagaaaggcggacaggtatccggtaagcggcagggtcggaacaggagagcgcacgagggagcttccagggggaaacgcctggtatctttatagtcctgtcgggtttcgccacctctgacttgagcgtcgatttttgtgatgctcgtcaggggggcggagcctatggaaaaacgccagcaacgcggcctttttacggttcctggccttttgctggccttttgctcacatgttctttcctgcgttatcccctgattctgtggataaccgtattaccgcctttgagtgagctgataccgctcgccgcagccgaacgaccgagcgcagcgagtcagtgagcgaggaagcggaagagcgcctgatgcggtattttctcc

SEQ ID NO: 36 - protein, 13 aa, Corynebacterium glutamicum
GGGSGGGGSGGGS

SEQ ID NO: 37 - DNA, 39 bp, Corynebacterium glutamicum
ggcggtggctctggaggtggtgggtccggcggtggctct

SEQ ID NO: 38 - DNA, 351 bp, Corynebacterium glutamicum
gtgcgtggcgagttttacaaagaaccccacatcatcaatgcctaaatggcgggtattttcatccaaacccaaccgcgcatcattccaatgctgatccaccccatccggataaaccaccatgaacggcaacggatcaaaagtcctgttggtgaagctgcgccccacagatcctgactgctgggagccatgaaaatagatcagcgcatccgtggtggaaccaaaaggctcaacaatacgaaacgttcgctttcggtcctgatgaaagagatgtccctgaatcatcatctaagtatgcattgtggtaagctcgaccaggacagtgccaccacaattttggaggattacaagaac